European Patent Application EP 4 394 041 A1, published July 3, 2024. Title: FUSION PROTEIN OF INTERLEUKIN-2 AND APPLICATION THEREOF IN IBD. Applicant: BEIJING VDJBIO CO., LTD. The sequence listing filed with the application follows.

SEQUENCE LISTING (5 sequences)

SEQ ID NO: 1 - protein, 133 aa, Homo sapiens
APTSSSTKKTQLQLEHLLLDLQMILNGINNYKNPKLTRMLTFKFYMPKKATELKHLQCLEEELKPLEEVLNLAQSKNFHLRPRDLISNINVIVLELKGSETTFMCEYADETATIVEFLNRWITFAQSIISTLT

SEQ ID NO: 2 - protein, 585 aa, Homo sapiens [sequence omitted]

SEQ ID NO: 3 - DNA, 2247 bp, synthetic construct
  source 1..2247: mol_type = other DNA
aagcttgccaccatgccactgctcctcctcctgcctctcctctgggctggtgctctggcagcaccaactagcagcagcactaagaagacccagctgcaactcgaacatctgctgctcgacctgcaaatgatcctgaatgggattaacaactataagaatcccaagctcactcggatgctcaccttcaagttctacatgcccaagaaagctactgaactcaaacatctgcaatgtctcgaagaggaactgaagccactggaagaggtgctgaatctggcccaatctaagaatttccacctgaggcctagggatctgataagcaatatcaacgtgattgtgctggagctgaagggttctgaaacaacctttatgtgtgagtacgcagacgaaaccgccaccatcgtcgagttcctcaatcggtggatcaccttcgctcagagcatcatctccacactcacaggaggcggtgggagtggtggtggagggtcagacgctcacaagagcgaggtggctcatcggttcaaagacctcggcgaggagaacttcaaggccctggtcctgatcgcctttgcccagtacctgcaacagtgtccctttgaagatcatgtcaagctcgtcaacgaggtgactgagttcgccaagacatgcgtcgcagacgagagtgccgagaattgcgacaaatccctccacaccctgtttggcgataagctctgtactgtcgctactctgagggagacatacggcgagatggctgactgctgcgccaagcaggagcccgagcggaatgaatgctttctgcaacacaaagacgacaatcctaatctgccaaggctcgtcagaccagaggtggatgtgatgtgtaccgcctttcatgataatgaggaaacctttctcaagaagtatctgtatgaaattgctagaaggcacccatacttctatgctcctgagctgctgttcttcgccaaacgctacaaggctgctttcactgaatgctgccaggcagccgacaaagcagcctgcctcctgccaaagctcgacgaactccgggacgaagggaaggcctcaagtgccaagcagagactgaagtgcgcaagcctccagaaattcggagaaagggcattcaaggcttgggcagtggcaaggctgtcccagaggtttcctaaggccgaatttgccgaagtctctaaactggtcacagacctgaccaaagtgcataccgaatgttgccacggcgacctcctggagtgcgctgacgatagggcagacctggccaaatacatttgcgagaaccaggatagtataagtagcaaactcaaggagtgctgtgagaagcctctcctggagaagtcccactgcatcgccgaagtggagaacgatgagatgccagctgacctccctagcctggcagccgactttgtcgaatcaaaggacgtctgcaagaattacgccgaggcaaaggatgtgttcctgggaatgtttctgtacgagtatgccagaaggcaccctgactattcagtcgtgctgctgctgcgcctggccaagacttatgaaactaccctggagaagtgttgcgcagctgccgacccacacgagtgttatgccaaggtgttcgatgagttcaagccactcgtcgaggagcctcagaacctgatcaagcagaactgcgaactcttcgagcagctgggagagtacaaattccagaacgccctgctggtgcggtacaccaagaaggtgccacaggtgtctacacctacactggttgaagtgtccagaaacctcggcaaggtgggaagcaaatgctgcaaacatcccgaggcaaagcggatgccatgcgcagaagattacctctctgtggtgctcaatcaactgtgcgtgctgcacgagaagacccccgtcagtgacagagtgaccaaatgctgcactgagagtctggtcaatagacggccatgcttcagtgccctggaggtggacgaaacatacgttcccaaagagttcaacgccgaaactttcacctttcatgctgacatttgtaccctgtcagagaaggagcggcagattaagaaacaaactgccctggtggaactggtgaaacacaagcctaaggcaaccaaagaacaactgaaggccgtcatggacgatttcgctgccttcgtcgagaagtgttgtaaggctgacgacaaggagacatgtttcgccgaagagggcaagaaactggttgctgccagccaagctgcactgggactgtga

SEQ ID NO: 4 - protein, 728 aa, Homo sapiens
APTSSSTKKTQLQLEHLLLDLQMILNGINNYKNPKLTRMLTFKFYMPKKATELKHLQCLEEELKPLEEVLNLAQSKNFHLRPRDLISNINVIVLELKGSETTFMCEYADETATIVEFLNRWITFAQSIISTLTGGGGSGGGGSDAHKSEVAHRFKDLGEENFKALVLIAFAQYLQQCPFEDHVKLVNEVTEFAKTCVADESAENCDKSLHTLFGDKLCTVATLRETYGEMADCCAKQEPERNECFLQHKDDNPNLPRLVRPEVDVMCTAFHDNEETFLKKYLYEIARRHPYFYAPELLFFAKRYKAAFTECCQAADKAACLLPKLDELRDEGKASSAKQRLKCASLQKFGERAFKAWAVARLSQRFPKAEFAEVSKLVTDLTKVHTECCHGDLLECADDRADLAKYICENQDSISSKLKECCEKPLLEKSHCIAEVENDEMPADLPSLAADFVESKDVCKNYAEAKDVFLGMFLYEYARRHPDYSVVLLLRLAKTYETTLEKCCAAADPHECYAKVFDEFKPLVEEPQNLIKQNCELFEQLGEYKFQNALLVRYTKKVPQVSTPTLVEVSRNLGKVGSKCCKHPEAKRMPCAEDYLSVVLNQLCVLHEKTPVSDRVTKCCTESLVNRRPCFSALEVDETYVPKEFNAETFTFHADICTLSEKERQIKKQTALVELVKHKPKATKEQLKAVMDDFAAFVEKCCKADDKETCFAEEGKKLVAASQAALGL

SEQ ID NO: 5 - DNA, 48 bp, synthetic construct
  source 1..48: mol_type = other DNA
atgccactgctcctcctcctgcctctcctctgggctggtgctctggca